European Patent Application EP 4 342 993 A1, published March 27, 2024. Title: Vaccine for HPV 6 and 11 infection. Applicant: DAIICHI SANKYO COMPANY, LIMITED. The sequence listing filed with the application follows.

SEQUENCE LISTING (20 sequences)

SEQ ID NO: 1 - DNA, 1154 bp, Artificial Sequence
  DNA fragment
gctagcgtaatacgactcactataaggagacccaagctacatttgcttctgacacaactgtgttcactagcaacctcaaacagacaccgccaccatggactggacctggatcctgttcctggtggccgccgccacaagagtgcacagcgaaagcgccaacgccagcaccagcgccaccaccatcgaccagctgtgcaagaccttcaacctgagcatgcacaccctgcagatcaactgcgtgttctgcaagaacgccctgaccaccgccgagatctacagctacgcctacaagcagctgaaggtgctgttcagaggcggctacccctacgccgcctgcgcctgcggactggaattccacggcaagatcaaccagtaccggcacttcgactacgccggctacgccaccacagtggaagaggaaacaaagcaggacatcctggacgtgctgatccggtgctacctgtgccacaagcccctgtgcgaggtggaaaaagtgaagcacatcctgaccaaggcccggttcatcaagctgaactgcacctggaaaggcagaggcctgcactgctggaccacctgcatggaagacatgctgcccagaggccggaagagaagaagccacggcagacacgtgaccctgaaggacatcgtgctggacctgcagccccccgaccccgtgggactgcacggatacggccagctggtggacagcagcgaggacgaggtggacgaagtggacggccaggacagccagccactgaagcagcactaccagatcgtgacctgctgctgcggctgcgacagcaacgtgcgactggtggtgcagtgcaccgagacagacatcagagaggtgcagcagctcctgctgggcaccctgaacatcgtgggccccatctgcgcccccaagacctgagctcgctttcttgctgtccaatttctattaaaggttcctttgttccctaagtccaactactaaactgggggatattatgaagggccttgagcatctggattctgcctaataaaaaacatttattttcattgcaaaaaaaaaaaaaaaaaaaaaaaaaaaaaaaaaaaaaaaaaaaaaaaaaaaaaaaaaaaaaaaaaaaaaaaaaaaaaaaaaaaaaaaaaaaaaaaaaaaaaagagcactagt

SEQ ID NO: 2 - DNA, 24 bp, Artificial Sequence
  sense primer
taatacgactcactataaggagac

SEQ ID NO: 3 - DNA, 129 bp, Artificial Sequence
  antisense primer
ttttttttttttttttttttttttttttttttttttttttttttttttttttttttttttttttttttttttttttttttttttttttttttttttttttgcaatgaaaataaatgttttttattaggc

SEQ ID NO: 4 - DNA, 1135 bp, Artificial Sequence
  template DNA
taatacgactcactataaggagacccaagctacatttgcttctgacacaactgtgttcactagcaacctcaaacagacaccgccaccatggactggacctggatcctgttcctggtggccgccgccacaagagtgcacagcgaaagcgccaacgccagcaccagcgccaccaccatcgaccagctgtgcaagaccttcaacctgagcatgcacaccctgcagatcaactgcgtgttctgcaagaacgccctgaccaccgccgagatctacagctacgcctacaagcagctgaaggtgctgttcagaggcggctacccctacgccgcctgcgcctgcggactggaattccacggcaagatcaaccagtaccggcacttcgactacgccggctacgccaccacagtggaagaggaaacaaagcaggacatcctggacgtgctgatccggtgctacctgtgccacaagcccctgtgcgaggtggaaaaagtgaagcacatcctgaccaaggcccggttcatcaagctgaactgcacctggaaaggcagaggcctgcactgctggaccacctgcatggaagacatgctgcccagaggccggaagagaagaagccacggcagacacgtgaccctgaaggacatcgtgctggacctgcagccccccgaccccgtgggactgcacggatacggccagctggtggacagcagcgaggacgaggtggacgaagtggacggccaggacagccagccactgaagcagcactaccagatcgtgacctgctgctgcggctgcgacagcaacgtgcgactggtggtgcagtgcaccgagacagacatcagagaggtgcagcagctcctgctgggcaccctgaacatcgtgggccccatctgcgcccccaagacctgagctcgctttcttgctgtccaatttctattaaaggttcctttgttccctaagtccaactactaaactgggggatattatgaagggccttgagcatctggattctgcctaataaaaaacatttattttcattgcaaaaaaaaaaaaaaaaaaaaaaaaaaaaaaaaaaaaaaaaaaaaaaaaaaaaaaaaaaaaaaaaaaaaaaaaaaaaaaaaaaaaaaaaaaaaaaaaaaaa

SEQ ID NO: 5 - RNA, 1118 nt, Artificial Sequence
  HPV E6-E7 fusion mRNA
aggagacccaagcuacauuugcuucugacacaacuguguucacuagcaaccucaaacagacaccgccaccauggacuggaccuggauccuguuccugguggccgccgccacaagagugcacagcgaaagcgccaacgccagcaccagcgccaccaccaucgaccagcugugcaagaccuucaaccugagcaugcacacccugcagaucaacugcguguucugcaagaacgcccugaccaccgccgagaucuacagcuacgccuacaagcagcugaaggugcuguucagaggcggcuaccccuacgccgccugcgccugcggacuggaauuccacggcaagaucaaccaguaccggcacuucgacuacgccggcuacgccaccacaguggaagaggaaacaaagcaggacauccuggacgugcugauccggugcuaccugugccacaagccccugugcgagguggaaaaagugaagcacauccugaccaaggcccgguucaucaagcugaacugcaccuggaaaggcagaggccugcacugcuggaccaccugcauggaagacaugcugcccagaggccggaagagaagaagccacggcagacacgugacccugaaggacaucgugcuggaccugcagccccccgaccccgugggacugcacggauacggccagcugguggacagcagcgaggacgagguggacgaaguggacggccaggacagccagccacugaagcagcacuaccagaucgugaccugcugcugcggcugcgacagcaacgugcgacugguggugcagugcaccgagacagacaucagagaggugcagcagcuccugcugggcacccugaacaucgugggccccaucugcgcccccaagaccugagcucgcuuucuugcuguccaauuucuauuaaagguuccuuuguucccuaaguccaacuacuaaacugggggauauuaugaagggccuugagcaucuggauucugccuaauaaaaaacauuuauuuucauugcaaaaaaaaaaaaaaaaaaaaaaaaaaaaaaaaaaaaaaaaaaaaaaaaaaaaaaaaaaaaaaaaaaaaaaaaaaaaaaaaaaaaaaaaaaaaaaaaaaaa

SEQ ID NO: 6 - DNA, 1154 bp, Artificial Sequence
  DNA fragment
gctagcgtaatacgactcactataaggagacccaagctacatttgcttctgacacaactgtgttcactagcaacctcaaacagacaccgccaccatggactggacctggatcctgttcctggtggccgccgccacaagagtgcacagcgagagcaaggacgccagcacaagcgccaccagcatcgaccagctgtgcaagaccttcaacctgagcctgcacaccctgcagatccagtgcgtgttctgcagaaacgccctgaccaccgccgagatctacgcctacgcctacaagaacctgaaggtcgtgtggcgggacaacttccccttcgccgcctgcgcctgcggcctggaactccagggaaagatcaaccagtaccggcacttcaactacgccgcctacgcccccacagtggaagaggaaacaaacgaggacatcctgaaggtgctgatccggtgctacctgtgccacaagcccctgtgcgagatcgagaagctgaagcacatcctgggcaaagcccggttcatcaagctgaacaaccagtggaaaggcagaggcctgcactgctggaccacctgcatggaagacctgctgcccagaggccggaagagaagaagccacggcagactggtcaccctgaaggacatcgtgctggacctgcagccccccgaccccgtgggactgcacggatacggccagctggaagacagcagcgaggacgaggtggacaaagtggacaagcaggacgcccagcccctgacacagcactaccagatcctgacctgctgctgcggctgcgacagcaacgtgcggctggtggtggaatgcaccgacggcgacatcagacagctgcaggacctgctcctgggcacactgaacatcgtgggccccatctgcgcccccaagccctgagctcgctttcttgctgtccaatttctattaaaggttcctttgttccctaagtccaactactaaactgggggatattatgaagggccttgagcatctggattctgcctaataaaaaacatttattttcattgcaaaaaaaaaaaaaaaaaaaaaaaaaaaaaaaaaaaaaaaaaaaaaaaaaaaaaaaaaaaaaaaaaaaaaaaaaaaaaaaaaaaaaaaaaaaaaaaaaaaaaagagcactagt

SEQ ID NO: 7 - DNA, 1135 bp, Artificial Sequence
  template DNA
taatacgactcactataaggagacccaagctacatttgcttctgacacaactgtgttcactagcaacctcaaacagacaccgccaccatggactggacctggatcctgttcctggtggccgccgccacaagagtgcacagcgagagcaaggacgccagcacaagcgccaccagcatcgaccagctgtgcaagaccttcaacctgagcctgcacaccctgcagatccagtgcgtgttctgcagaaacgccctgaccaccgccgagatctacgcctacgcctacaagaacctgaaggtcgtgtggcgggacaacttccccttcgccgcctgcgcctgcggcctggaactccagggaaagatcaaccagtaccggcacttcaactacgccgcctacgcccccacagtggaagaggaaacaaacgaggacatcctgaaggtgctgatccggtgctacctgtgccacaagcccctgtgcgagatcgagaagctgaagcacatcctgggcaaagcccggttcatcaagctgaacaaccagtggaaaggcagaggcctgcactgctggaccacctgcatggaagacctgctgcccagaggccggaagagaagaagccacggcagactggtcaccctgaaggacatcgtgctggacctgcagccccccgaccccgtgggactgcacggatacggccagctggaagacagcagcgaggacgaggtggacaaagtggacaagcaggacgcccagcccctgacacagcactaccagatcctgacctgctgctgcggctgcgacagcaacgtgcggctggtggtggaatgcaccgacggcgacatcagacagctgcaggacctgctcctgggcacactgaacatcgtgggccccatctgcgcccccaagccctgagctcgctttcttgctgtccaatttctattaaaggttcctttgttccctaagtccaactactaaactgggggatattatgaagggccttgagcatctggattctgcctaataaaaaacatttattttcattgcaaaaaaaaaaaaaaaaaaaaaaaaaaaaaaaaaaaaaaaaaaaaaaaaaaaaaaaaaaaaaaaaaaaaaaaaaaaaaaaaaaaaaaaaaaaaaaaaaaaa

SEQ ID NO: 8 - RNA, 1118 nt, Artificial Sequence
  HPV11 E6-E7 fusion mRNA
aggagacccaagcuacauuugcuucugacacaacuguguucacuagcaaccucaaacagacaccgccaccauggacuggaccuggauccuguuccugguggccgccgccacaagagugcacagcgagagcaaggacgccagcacaagcgccaccagcaucgaccagcugugcaagaccuucaaccugagccugcacacccugcagauccagugcguguucugcagaaacgcccugaccaccgccgagaucuacgccuacgccuacaagaaccugaaggucguguggcgggacaacuuccccuucgccgccugcgccugcggccuggaacuccagggaaagaucaaccaguaccggcacuucaacuacgccgccuacgcccccacaguggaagaggaaacaaacgaggacauccugaaggugcugauccggugcuaccugugccacaagccccugugcgagaucgagaagcugaagcacauccugggcaaagcccgguucaucaagcugaacaaccaguggaaaggcagaggccugcacugcuggaccaccugcauggaagaccugcugcccagaggccggaagagaagaagccacggcagacuggucacccugaaggacaucgugcuggaccugcagccccccgaccccgugggacugcacggauacggccagcuggaagacagcagcgaggacgagguggacaaaguggacaagcaggacgcccagccccugacacagcacuaccagauccugaccugcugcugcggcugcgacagcaacgugcggcuggugguggaaugcaccgacggcgacaucagacagcugcaggaccugcuccugggcacacugaacaucgugggccccaucugcgcccccaagcccugagcucgcuuucuugcuguccaauuucuauuaaagguuccuuuguucccuaaguccaacuacuaaacugggggauauuaugaagggccuugagcaucuggauucugccuaauaaaaaacauuuauuuucauugcaaaaaaaaaaaaaaaaaaaaaaaaaaaaaaaaaaaaaaaaaaaaaaaaaaaaaaaaaaaaaaaaaaaaaaaaaaaaaaaaaaaaaaaaaaaaaaaaaaaa

SEQ ID NO: 9 - DNA, 1934 bp, Artificial Sequence
  DNA fragment
gctagcgtaatacgactcactataaggagacccaagctacatttgcttctgacacaactgtgttcactagcaacctcaaacagacaccgccaccatggactggacctggatcctgttcctggtggccgccgccacaagagtgcacagcgaaagcgccaacgccagcaccagcgccaccaccatcgaccagctgtgcaagaccttcaacctgagcatgcacaccctgcagatcaactgcgtgttctgcaagaacgccctgaccaccgccgagatctacagctacgcctacaagcagctgaaggtgctgttcagaggcggctacccctacgccgcctgcgcctgcggactggaattccacggcaagatcaaccagtaccggcacttcgactacgccggctacgccaccacagtggaagaggaaacaaagcaggacatcctggacgtgctgatccggtgctacctgtgccacaagcccctgtgcgaggtggaaaaagtgaagcacatcctgaccaaggcccggttcatcaagctgaactgcacctggaaaggcagaggcctgcactgctggaccacctgcatggaagacatgctgcccagaggccggaagagaagaagccacggcagacacgtgaccctgaaggacatcgtgctggacctgcagccccccgaccccgtgggactgcacggatacggccagctggtggacagcagcgaggacgaggtggacgaagtggacggccaggacagccagccactgaagcagcactaccagatcgtgacctgctgctgcggctgcgacagcaacgtgcgactggtggtgcagtgcaccgagacagacatcagagaggtgcagcagctcctgctgggcaccctgaacatcgtgggccccatctgcgcccccaagaccagaggaagaaagcggagaagcgagagcaaggacgccagcaccagcgccaccagcatcgaccagctctgcaaaaccttcaacctgagcctgcacacactccagatccagtgcgtgttctgccggaacgccctgacaacagccgaaatctacgcctacgcctacaagaacctgaaggtcgtgtggcgggacaacttccccttcgccgcctgcgcctgcggcctcgagctgcagggaaaaatcaaccagtacagacacttcaactacgccgcctacgcccccaccgtcgaggaagagacaaacgaggacatcctgaaggtcctcatccgctgctacctgtgccacaaacccctctgcgagatcgagaagctgaaacacatcctgggcaaagcccgcttcatcaagctcaacaaccagtggaaaggccggggactccactgctggacaacatgcatggaagacctgctcccccggggcagaaagaggcgcagccacggaaggctggtcacactgaaagacatcgtcctggacctccagccaccggacccagtcggcctgcacggctacggacagctcgaggacagcagcgaggacgaagtggacaaggtggacaagcaggacgcccagcccctgacccagcactaccagatcctgacatgctgctgcggctgcgacagcaacgtgcggctggtcgtggaatgcaccgacggcgacatcagacagctgcaggacctgctcctgggaacactgaacatcgtgggacccatctgcgcccccaagccctgagctcgctttcttgctgtccaatttctattaaaggttcctttgttccctaagtccaactactaaactgggggatattatgaagggccttgagcatctggattctgcctaataaaaaacatttattttcattgcaaaaaaaaaaaaaaaaaaaaaaaaaaaaaaaaaaaaaaaaaaaaaaaaaaaaaaaaaaaaaaaaaaaaaaaaaaaaaaaaaaaaaaaaaaaaaaaaaaaaaagagcactagt

SEQ ID NO: 10 - DNA, 1915 bp, Artificial Sequence
  template DNA
taatacgactcactataaggagacccaagctacatttgcttctgacacaactgtgttcactagcaacctcaaacagacaccgccaccatggactggacctggatcctgttcctggtggccgccgccacaagagtgcacagcgaaagcgccaacgccagcaccagcgccaccaccatcgaccagctgtgcaagaccttcaacctgagcatgcacaccctgcagatcaactgcgtgttctgcaagaacgccctgaccaccgccgagatctacagctacgcctacaagcagctgaaggtgctgttcagaggcggctacccctacgccgcctgcgcctgcggactggaattccacggcaagatcaaccagtaccggcacttcgactacgccggctacgccaccacagtggaagaggaaacaaagcaggacatcctggacgtgctgatccggtgctacctgtgccacaagcccctgtgcgaggtggaaaaagtgaagcacatcctgaccaaggcccggttcatcaagctgaactgcacctggaaaggcagaggcctgcactgctggaccacctgcatggaagacatgctgcccagaggccggaagagaagaagccacggcagacacgtgaccctgaaggacatcgtgctggacctgcagccccccgaccccgtgggactgcacggatacggccagctggtggacagcagcgaggacgaggtggacgaagtggacggccaggacagccagccactgaagcagcactaccagatcgtgacctgctgctgcggctgcgacagcaacgtgcgactggtggtgcagtgcaccgagacagacatcagagaggtgcagcagctcctgctgggcaccctgaacatcgtgggccccatctgcgcccccaagaccagaggaagaaagcggagaagcgagagcaaggacgccagcaccagcgccaccagcatcgaccagctctgcaaaaccttcaacctgagcctgcacacactccagatccagtgcgtgttctgccggaacgccctgacaacagccgaaatctacgcctacgcctacaagaacctgaaggtcgtgtggcgggacaacttccccttcgccgcctgcgcctgcggcctcgagctgcagggaaaaatcaaccagtacagacacttcaactacgccgcctacgcccccaccgtcgaggaagagacaaacgaggacatcctgaaggtcctcatccgctgctacctgtgccacaaacccctctgcgagatcgagaagctgaaacacatcctgggcaaagcccgcttcatcaagctcaacaaccagtggaaaggccggggactccactgctggacaacatgcatggaagacctgctcccccggggcagaaagaggcgcagccacggaaggctggtcacactgaaagacatcgtcctggacctccagccaccggacccagtcggcctgcacggctacggacagctcgaggacagcagcgaggacgaagtggacaaggtggacaagcaggacgcccagcccctgacccagcactaccagatcctgacatgctgctgcggctgcgacagcaacgtgcggctggtcgtggaatgcaccgacggcgacatcagacagctgcaggacctgctcctgggaacactgaacatcgtgggacccatctgcgcccccaagccctgagctcgctttcttgctgtccaatttctattaaaggttcctttgttccctaagtccaactactaaactgggggatattatgaagggccttgagcatctggattctgcctaataaaaaacatttattttcattgcaaaaaaaaaaaaaaaaaaaaaaaaaaaaaaaaaaaaaaaaaaaaaaaaaaaaaaaaaaaaaaaaaaaaaaaaaaaaaaaaaaaaaaaaaaaaaaaaaaaa

SEQ ID NO: 11 - RNA, 1898 nt, Artificial Sequence
  HPV6 E6-E7 HPV11 E6-E7 fusion mRNA
aggagacccaagcuacauuugcuucugacacaacuguguucacuagcaaccucaaacagacaccgccaccauggacuggaccuggauccuguuccugguggccgccgccacaagagugcacagcgaaagcgccaacgccagcaccagcgccaccaccaucgaccagcugugcaagaccuucaaccugagcaugcacacccugcagaucaacugcguguucugcaagaacgcccugaccaccgccgagaucuacagcuacgccuacaagcagcugaaggugcuguucagaggcggcuaccccuacgccgccugcgccugcggacuggaauuccacggcaagaucaaccaguaccggcacuucgacuacgccggcuacgccaccacaguggaagaggaaacaaagcaggacauccuggacgugcugauccggugcuaccugugccacaagccccugugcgagguggaaaaagugaagcacauccugaccaaggcccgguucaucaagcugaacugcaccuggaaaggcagaggccugcacugcuggaccaccugcauggaagacaugcugcccagaggccggaagagaagaagccacggcagacacgugacccugaaggacaucgugcuggaccugcagccccccgaccccgugggacugcacggauacggccagcugguggacagcagcgaggacgagguggacgaaguggacggccaggacagccagccacugaagcagcacuaccagaucgugaccugcugcugcggcugcgacagcaacgugcgacugguggugcagugcaccgagacagacaucagagaggugcagcagcuccugcugggcacccugaacaucgugggccccaucugcgcccccaagaccagaggaagaaagcggagaagcgagagcaaggacgccagcaccagcgccaccagcaucgaccagcucugcaaaaccuucaaccugagccugcacacacuccagauccagugcguguucugccggaacgcccugacaacagccgaaaucuacgccuacgccuacaagaaccugaaggucguguggcgggacaacuuccccuucgccgccugcgccugcggccucgagcugcagggaaaaaucaaccaguacagacacuucaacuacgccgccuacgcccccaccgucgaggaagagacaaacgaggacauccugaagguccucauccgcugcuaccugugccacaaaccccucugcgagaucgagaagcugaaacacauccugggcaaagcccgcuucaucaagcucaacaaccaguggaaaggccggggacuccacugcuggacaacaugcauggaagaccugcucccccggggcagaaagaggcgcagccacggaaggcuggucacacugaaagacaucguccuggaccuccagccaccggacccagucggccugcacggcuacggacagcucgaggacagcagcgaggacgaaguggacaagguggacaagcaggacgcccagccccugacccagcacuaccagauccugacaugcugcugcggcugcgacagcaacgugcggcuggucguggaaugcaccgacggcgacaucagacagcugcaggaccugcuccugggaacacugaacaucgugggacccaucugcgcccccaagcccugagcucgcuuucuugcuguccaauuucuauuaaagguuccuuuguucccuaaguccaacuacuaaacugggggauauuaugaagggccuugagcaucuggauucugccuaauaaaaaacauuuauuuucauugcaaaaaaaaaaaaaaaaaaaaaaaaaaaaaaaaaaaaaaaaaaaaaaaaaaaaaaaaaaaaaaaaaaaaaaaaaaaaaaaaaaaaaaaaaaaaaaaaaaaa

SEQ ID NO: 12 - protein, 149 aa, Human papillomavirus type 6
ESANASTSATTIDQLCKTFNLSMHTLQINCVFCKNALTTAEIYSYAYKQLKVLFRGGYPYAACACGLEFHGKINQYRHFDYAGYATTVEEETKQDILDVLIRCYLCHKPLCEVEKVKHILTKARFIKLNCTWKGRGLHCWTTCMEDMLP

SEQ ID NO: 13 - protein, 97 aa, Human papillomavirus type 6
HGRHVTLKDIVLDLQPPDPVGLHGYGQLVDSSEDEVDEVDGQDSQPLKQHYQIVTCCCGCDSNVRLVVQCTETDIREVQQLLLGTLNIVGPICAPKT

SEQ ID NO: 14 - protein, 149 aa, Human papillomavirus type 11
ESKDASTSATSIDQLCKTFNLSLHTLQIQCVFCRNALTTAEIYAYAYKNLKVVWRDNFPFAACACGLELQGKINQYRHFNYAAYAPTVEEETNEDILKVLIRCYLCHKPLCEIEKLKHILGKARFIKLNNQWKGRGLHCWTTCMEDLLP

SEQ ID NO: 15 - protein, 97 aa, Human papillomavirus type 11
HGRLVTLKDIVLDLQPPDPVGLHGYGQLEDSSEDEVDKVDKQDAQPLTQHYQILTCCCGCDSNVRLVVECTDGDIRQLQDLLLGTLNIVGPICAPKP

SEQ ID NO: 16 - protein, 7 aa, Artificial Sequence
  proteolytic cleavage site
RGRKRRS

SEQ ID NO: 17 - protein, 253 aa, Artificial Sequence
  fusion protein of E6 and E7 antigens from human papillomavirus type 6
ESANASTSATTIDQLCKTFNLSMHTLQINCVFCKNALTTAEIYSYAYKQLKVLFRGGYPYAACACGLEFHGKINQYRHFDYAGYATTVEEETKQDILDVLIRCYLCHKPLCEVEKVKHILTKARFIKLNCTWKGRGLHCWTTCMEDMLPRGRKRRSHGRHVTLKDIVLDLQPPDPVGLHGYGQLVDSSEDEVDEVDGQDSQPLKQHYQIVTCCCGCDSNVRLVVQCTETDIREVQQLLLGTLNIVGPICAPKT

SEQ ID NO: 18 - protein, 253 aa, Artificial Sequence
  fusion protein of E6 and E7 antigens from human papillomavirus type 11
ESKDASTSATSIDQLCKTFNLSLHTLQIQCVFCRNALTTAEIYAYAYKNLKVVWRDNFPFAACACGLELQGKINQYRHFNYAAYAPTVEEETNEDILKVLIRCYLCHKPLCEIEKLKHILGKARFIKLNNQWKGRGLHCWTTCMEDLLPRGRKRRSHGRLVTLKDIVLDLQPPDPVGLHGYGQLEDSSEDEVDKVDKQDAQPLTQHYQILTCCCGCDSNVRLVVECTDGDIRQLQDLLLGTLNIVGPICAPKP

SEQ ID NO: 19 - protein, 513 aa, Artificial Sequence
  fusion protein of E6 and E7 antigens from human papillomavirus type 6 and type 11
ESANASTSATTIDQLCKTFNLSMHTLQINCVFCKNALTTAEIYSYAYKQLKVLFRGGYPYAACACGLEFHGKINQYRHFDYAGYATTVEEETKQDILDVLIRCYLCHKPLCEVEKVKHILTKARFIKLNCTWKGRGLHCWTTCMEDMLPRGRKRRSHGRHVTLKDIVLDLQPPDPVGLHGYGQLVDSSEDEVDEVDGQDSQPLKQHYQIVTCCCGCDSNVRLVVQCTETDIREVQQLLLGTLNIVGPICAPKTRGRKRRSESKDASTSATSIDQLCKTFNLSLHTLQIQCVFCRNALTTAEIYAYAYKNLKVVWRDNFPFAACACGLELQGKINQYRHFNYAAYAPTVEEETNEDILKVLIRCYLCHKPLCEIEKLKHILGKARFIKLNNQWKGRGLHCWTTCMEDLLPRGRKRRSHGRLVTLKDIVLDLQPPDPVGLHGYGQLEDSSEDEVDKVDKQDAQPLTQHYQILTCCCGCDSNVRLVVECTDGDIRQLQDLLLGTLNIVGPICAPKP

SEQ ID NO: 20 - protein, 18 aa, Artificial Sequence
  IgE leader sequence
MDWTWILFLVAAATRVHS